European Patent Application EP 4 653 466 A1, published November 26, 2025. Title: ANTI-ALK-1 ANTIBODY AND USE THEREOF. Applicant: KINTOR PHARMACEUTICAL (GUANGDONG) CO., LTD. The sequence listing filed with the application follows.

SEQUENCE LISTING (94 sequences)

SEQ ID NO: 1 - protein, 118 aa, synthetic construct
QVQLQESGPGLVKPSQTLSLTCTVSGGSISSGEYYWNWIRQHPGKGLEWIGYIYYSGSTYYNPSLKSRVTISVDTSKNQFSLKLSSVTAADTAVYYCARESVAGFDYWGQGTLVTVSS

SEQ ID NO: 2 - protein, 10 aa, synthetic construct
GGSISSGEYY

SEQ ID NO: 3 - protein, 7 aa, synthetic construct
IYYSGST

SEQ ID NO: 4 - protein, 10 aa, synthetic construct
ARESVAGFDY

SEQ ID NO: 5 - protein, 108 aa, synthetic construct
EIVLTQSPGTLSLSPGERATLSCRASQSVSSSYLAWYQQKPGQAPRLLIYGTSSRATGIPDRFSGSGSGTDFTLTISRLEPEDFAVYYCQQYGSSPITFGQGTRLEIK

SEQ ID NO: 6 - protein, 7 aa, synthetic construct
QSVSSSY

SEQ ID NO: 7 - skipped

SEQ ID NO: 8 - protein, 9 aa, synthetic construct
QQYGSSPIT

SEQ ID NO: 9 - protein, 329 aa, synthetic construct
ASTKGPSVFPLAPSSKSTSGGTAALGCLVKDYFPEPVTVSWNSGALTSGVHTFPAVLQSSGLYSLSSVVTVPSSSLGTQTYICNVNHKPSNTKVDKKVEPKSCDKTHTCPPCPAPEAAGGPSVFLFPPKPKDTLMISRTPEVTCVVVDVSHEDPEVKFNWYVDGVEVHNAKTKPREEQYNSTYRVVSVLTVLHQDWLNGKEYKCKVSNKALPAPIEKTISKAKGQPREPQVYTLPPSREEMTKNQVSLTCLVKGFYPSDIAVEWESNGQPENNYKTTPPVLDSDGSFFLYSKLTVDKSRWQQGNVFSCSVMHEALHNHYTQKSLSLSPG

SEQ ID NO: 10 - protein, 107 aa, synthetic construct [sequence omitted]

SEQ ID NO: 11 - protein, 108 aa, synthetic construct
EIVLTQSPGTLSLSPGERATLSCRASQSVSSSYLAWYQQKPGQAPRLLIYGTSSRATGIPDRFSGSGSGTDFTLTISRLEPEDFAVYYCQAYGSWPITFGQGTRLEIK

SEQ ID NO: 12 - protein, 9 aa, synthetic construct
QAYGSWPIT

SEQ ID NO: 13 - protein, 108 aa, synthetic construct
EIVLTQSPGTLSLSPGERATLSCRASQSVSSSYLAWYQQKPGQAPRLLIYGTSSRATGIPDRFSGSGSGTDFTLTISRLEPEDFAVYYCQLYGSFPITFGQGTRLEIK

SEQ ID NO: 14 - protein, 9 aa, synthetic construct
QLYGSFPIT

SEQ ID NO: 15 - protein, 108 aa, synthetic construct
EIVLTQSPGTLSLSPGERATLSCRASQSVSSSYLAWYQQKPGQAPRLLIYGTSSRATGIPDRFSGSGSGTDFTLTISRLEPEDFAVYYCQGYGSFPITFGQGTRLEIK

SEQ ID NO: 16 - protein, 9 aa, synthetic construct
QGYGSFPIT

SEQ ID NO: 17 - protein, 108 aa, synthetic construct
EIVLTQSPGTLSLSPGERATLSCRASQSVSSSYLAWYQQKPGQAPRLLIYGTSSRATGIPDRFSGSGSGTDFTLTISRLEPEDFAVYYCQFYGSFPITFGQGTRLEIK

SEQ ID NO: 18 - protein, 9 aa, synthetic construct
QFYGSFPIT

SEQ ID NO: 19 - protein, 108 aa, synthetic construct
EIVLTQSPGTLSLSPGERATLSCRASQSVSSSYLAWYQQKPGQAPRLLIYGTSSRATGIPDRFSGSGSGTDFTLTISRLEPEDFAVYYCQPYGSVPITFGQGTRLEIK

SEQ ID NO: 20 - protein, 9 aa, synthetic construct
QPYGSVPIT

SEQ ID NO: 21 - protein, 108 aa, synthetic construct
EIVLTQSPGTLSLSPGERATLSCRASQSVSSSYLAWYQQKPGQAPRLLIYGTSSRATGIPDRFSGSGSGTDFTLTISRLEPEDFAVYYCQAYGSVPITFGQGTRLEIK

SEQ ID NO: 22 - protein, 9 aa, synthetic construct
QAYGSVPIT

SEQ ID NO: 23 - protein, 108 aa, synthetic construct
EIVLTQSPGTLSLSPGERATLSCRASQSVSSSYLAWYQQKPGQAPRLLIYGTSSRATGIPDRFSGSGSGTDFTLTISRLEPEDFAVYYCQMYGSIPITFGQGTRLEIK

SEQ ID NO: 24 - protein, 9 aa, synthetic construct
QMYGSIPIT

SEQ ID NO: 25 - protein, 108 aa, synthetic construct
EIVLTQSPGTLSLSPGERATLSCRASQSVSSSYLAWYQQKPGQAPRLLIYGTSSRATGIPDRFSGSGSGTDFTLTISRLEPEDFAVYYCQIYGSWPITFGQGTRLEIK

SEQ ID NO: 26 - protein, 9 aa, synthetic construct
QIYGSWPIT

SEQ ID NO: 27 - protein, 108 aa, synthetic construct
EIVLTQSPGTLSLSPGERATLSCRASQSVSSSYLAWYQQKPGQAPRLLIYGTSSRATGIPDRFSGSGSGTDFTLTISRLEPEDFAVYYCQIYGSIPITFGQGTRLEIK

SEQ ID NO: 28 - protein, 9 aa, synthetic construct
QIYGSIPIT

SEQ ID NO: 29 - protein, 108 aa, synthetic construct
EIVLTQSPGTLSLSPGERATLSCRASQSVSSSYLAWYQQKPGQAPRLLIYGTSSRATGIPDRFSGSGSGTDFTLTISRLEPEDFAVYYCQPYGSIPITFGQGTRLEIK

SEQ ID NO: 30 - protein, 9 aa, synthetic construct
QPYGSIPIT

SEQ ID NO: 31 - protein, 108 aa, synthetic construct
EIVLTQSPGTLSLSPGERATLSCRASQSVSSSYLAWYQQKPGQAPRLLIYGTSSRATGIPDRFSGSGSGTDFTLTISRLEPEDFAVYYCQMYGSWPITFGQGTRLEIK

SEQ ID NO: 32 - protein, 9 aa, synthetic construct
QMYGSWPIT

SEQ ID NO: 33 - protein, 108 aa, synthetic construct
EIVLTQSPGTLSLSPGERATLSCRASQSVSSSYLAWYQQKPGQAPRLLIYGTSSRATGIPDRFSGSGSGTDFTLTISRLEPEDFAVYYCQWYGSVPITFGQGTRLEIK

SEQ ID NO: 34 - protein, 9 aa, synthetic construct
QWYGSVPIT

SEQ ID NO: 35 - protein, 108 aa, synthetic construct
EIVLTQSPGTLSLSPGERATLSCRASQSVSSSYLAWYQQKPGQAPRLLIYGTSSRATGIPDRFSGSGSGTDFTLTISRLEPEDFAVYYCQVYGSIPITFGQGTRLEIK

SEQ ID NO: 36 - protein, 9 aa, synthetic construct
QVYGSIPIT

SEQ ID NO: 37 - protein, 108 aa, synthetic construct
EIVLTQSPGTLSLSPGERATLSCRASQSVSSSYLAWYQQKPGQAPRLLIYGTSSRATGIPDRFSGSGSGTDFTLTISRLEPEDFAVYYCQGYGSIPITFGQGTRLEIK

SEQ ID NO: 38 - protein, 9 aa, synthetic construct
QGYGSIPIT

SEQ ID NO: 39 - protein, 108 aa, synthetic construct
EIVLTQSPGTLSLSPGERATLSCRASQSVSSSYLAWYQQKPGQAPRLLIYGTSSRATGIPDRFSGSGSGTDFTLTISRLEPEDFAVYYCQFYGSWPITFGQGTRLEIK

SEQ ID NO: 40 - protein, 9 aa, synthetic construct
QFYGSWPIT

SEQ ID NO: 41 - protein, 108 aa, synthetic construct
EIVLTQSPGTLSLSPGERATLSCRASQSVSSSYLAWYQQKPGQAPRLLIYGTSSRATGIPDRFSGSGSGTDFTLTISRLEPEDFAVYYCQFYGSVPITFGQGTRLEIK

SEQ ID NO: 42 - protein, 9 aa, synthetic construct
QFYGSVPIT

SEQ ID NO: 43 - protein, 108 aa, synthetic construct
EIVLTQSPGTLSLSPGERATLSCRASQSVSSSYLAWYQQKPGQAPRLLIYGTSSRATGIPDRFSGSGSGTDFTLTISRLEPEDFAVYYCQFYGSIPITFGQGTRLEIK

SEQ ID NO: 44 - protein, 9 aa, synthetic construct
QFYGSIPIT

SEQ ID NO: 45 - protein, 108 aa, synthetic construct
EIVLTQSPGTLSLSPGERATLSCRASQSVSSSYLAWYQQKPGQAPRLLIYGTSSRATGIPDRFSGSGSGTDFTLTISRLEPEDFAVYYCQVYGSWPITFGQGTRLEIK

SEQ ID NO: 46 - protein, 9 aa, synthetic construct
QVYGSWPIT

SEQ ID NO: 47 - protein, 108 aa, synthetic construct
EIVLTQSPGTLSLSPGERATLSCRASQSVSSSYLAWYQQKPGQAPRLLIYGTSSRATGIPDRFSGSGSGTDFTLTISRLEPEDFAVYYCQVYGSVPITFGQGTRLEIK

SEQ ID NO: 48 - protein, 9 aa, synthetic construct
QVYGSVPIT

SEQ ID NO: 49 - protein, 108 aa, synthetic construct
EIVLTQSPGTLSLSPGERATLSCRASQSVSSSYLAWYQQKPGQAPRLLIYGTSSRATGIPDRFSGSGSGTDFTLTISRLEPEDFAVYYCQGYGSWPITFGQGTRLEIK

SEQ ID NO: 50 - protein, 9 aa, synthetic construct
QGYGSWPIT

SEQ ID NO: 51 - protein, 108 aa, synthetic construct
EIVLTQSPGTLSLSPGERATLSCRASQSVSSSYLAWYQQKPGQAPRLLIYGTSSRATGIPDRFSGSGSGTDFTLTISRLEPEDFAVYYCQIYGSVPITFGQGTRLEIK

SEQ ID NO: 52 - protein, 9 aa, synthetic construct
QIYGSVPIT

SEQ ID NO: 53 - protein, 108 aa, synthetic construct
EIVLTQSPGTLSLSPGERATLSCRASQSVSSSYLAWYQQKPGQAPRLLIYGTSSRATGIPDRFSGSGSGTDFTLTISRLEPEDFAVYYCQPYGSWPITFGQGTRLEIK

SEQ ID NO: 54 - protein, 9 aa, synthetic construct
QPYGSWPIT

SEQ ID NO: 55 - protein, 108 aa, synthetic construct
EIVLTQSPGTLSLSPGERATLSCRASQSVSSSYLAWYQQKPGQAPRLLIYGTSSRATGIPDRFSGSGSGTDFTLTISRLEPEDFAVYYCQGYGSVPITFGQGTRLEIK

SEQ ID NO: 56 - protein, 9 aa, synthetic construct
QGYGSVPIT

SEQ ID NO: 57 - protein, 123 aa, synthetic construct [sequence omitted]

SEQ ID NO: 58 - protein, 8 aa, synthetic construct
GYTFTNYG

SEQ ID NO: 59 - protein, 8 aa, synthetic construct
INTYTGEP

SEQ ID NO: 60 - protein, 16 aa, synthetic construct
AKYPHYYGSSHWYFDV

SEQ ID NO: 61 - protein, 107 aa, synthetic construct [sequence omitted]

SEQ ID NO: 62 - protein, 6 aa, synthetic construct
QDISNY

SEQ ID NO: 63 - skipped

SEQ ID NO: 64 - protein, 9 aa, synthetic construct
QQYSTVPWT

SEQ ID NO: 65 - protein, 20 aa, synthetic construct
GGGGSGGGGSGGGGSGGGGS

SEQ ID NO: 66 - protein, 108 aa, synthetic construct
EIVLTQSPGTLSLSPGERATLSCRASQSVSSSYLAWYQQKPGQAPRLLIYGTSSRATGIPDRFSGSGSGTDFTLTISRLEPEDFAVYYCQAYGSWPITFGCGTRLEIK

SEQ ID NO: 67 - protein, 118 aa, synthetic construct
QVQLQESGPGLVKPSQTLSLTCTVSGGSISSGEYYWNWIRQHPGKCLEWIGYIYYSGSTYYNPSLKSRVTISVDTSKNQFSLKLSSVTAADTAVYYCARESVAGFDYWGQGTLVTVSS

SEQ ID NO: 68 - protein, 718 aa, synthetic construct
EVQLVESGGGLVQPGGSLRLSCAASGYTFTNYGMNWVRQAPGKGLEWVGWINTYTGEPTYAADFKRRFTFSLDTSKSTAYLQMNSLRAEDTAVYYCAKYPHYYGSSHWYFDVWGQGTLVTVSSASTKGPSVFPLAPSSKSTSGGTAALGCLVKDYFPEPVTVSWNSGALTSGVHTFPAVLQSSGLYSLSSVVTVPSSSLGTQTYICNVNHKPSNTKVDKKVEPKSCDKTHTCPPCPAPEAAGGPSVFLFPPKPKDTLMISRTPEVTCVVVDVSHEDPEVKFNWYVDGVEVHNAKTKPREEQYNSTYRVVSVLTVLHQDWLNGKEYKCKVSNKALPAPIEKTISKAKGQPREPQVYTLPPSREEMTKNQVSLTCLVKGFYPSDIAVEWESNGQPENNYKTTPPVLDSDGSFFLYSKLTVDKSRWQQGNVFSCSVMHEALHNHYTQKSLSLSPGGGGGSGGGGSGGGGSGGGGSQVQLQESGPGLVKPSQTLSLTCTVSGGSISSGEYYWNWIRQHPGKCLEWIGYIYYSGSTYYNPSLKSRVTISVDTSKNQFSLKLSSVTAADTAVYYCARESVAGFDYWGQGTLVTVSSGGGGSGGGGSGGGGSGGGGSEIVLTQSPGTLSLSPGERATLSCRASQSVSSSYLAWYQQKPGQAPRLLIYGTSSRATGIPDRFSGSGSGTDFTLTISRLEPEDFAVYYCQAYGSWPITFGCGTRLEIK

SEQ ID NO: 69 - protein, 214 aa, synthetic construct
DIQMTQSPSSLSASVGDRVTITCSASQDISNYLNWYQQKPGKAPKVLIYFTSSLHSGVPSRFSGSGSGTDFTLTISSLQPEDFATYYCQQYSTVPWTFGQGTKVEIKRTVAAPSVFIFPPSDEQLKSGTASVVCLLNNFYPREAKVQWKVDNALQSGNSQESVTEQDSKDSTYSLSSTLTLSKADYEKHKVYACEVTHQGLSSPVTKSFNRGEC

SEQ ID NO: 70 - protein, 118 aa, synthetic construct
QVQLQESGPGLVKPSQTLSLTCTVSGGSISSGEYYWNWIRQHPGCGLEWIGYIYYSGSTYYNPSLKSRVTISVDTSKNQFSLKLSSVTAADTAVYYCARESVAGFDYWGQGTLVTVSS

SEQ ID NO: 71 - protein, 108 aa, synthetic construct
EIVLTQSPGTLSLSPGERATLSCRASQSVSSSYLAWYQQKPGQAPRLLIYGTSSRATGIPDRFSGSGSGTDFTLTISRLEPEDFAVYYCQAYGSWPITFCQGTRLEIK

SEQ ID NO: 72 - protein, 108 aa, synthetic construct
EIVLTQSPGTLSLSPGERATLSCRASQSVSSSYLAWYQQKPGQAPRLLIYGTSSRATGIPDRFSGSGSGTDFTLTISRLEPEDFAVYYCQAYGSWPITFGQCTRLEIK

SEQ ID NO: 73 - protein, 118 aa, synthetic construct
QVQLQESGPGLVKPSQTLSLTCTVSGGSISSGEYYWNWIRQHPGKGCEWIGYIYYSGSTYYNPSLKSRVTISVDTSKNQFSLKLSSVTAADTAVYYCARESVAGFDYWGQGTLVTVSS

SEQ ID NO: 74 - protein, 108 aa, synthetic construct
EIVLTQSPGTLSLSPGERATLSCRASQSVSSSYLAWYQQKPGQAPRLLIYGTSSRATGIPDRFSGSGSGTDFTLTISRLEPEDFAVYYCQAYGSWPITCGQGTRLEIK

SEQ ID NO: 75 - protein, 118 aa, synthetic construct
QVQLQESGPGLVKPSQTLSLTCTVSGGSISSGEYYWNWIRQHPGKGLEWIGYIYYSGSTYYNPSLKSRVTISVDTSKNQFSLKLSSVTAADTAVYYCARESVAGFDYWGCGTLVTVSS

SEQ ID NO: 76 - protein, 108 aa, synthetic construct
EIVLTQSPGTLSLSPGERATLSCRASQSVSSSYLAWYQQKPGQCPRLLIYGTSSRATGIPDRFSGSGSGTDFTLTISRLEPEDFAVYYCQAYGSWPITFGQGTRLEIK

SEQ ID NO: 77 - protein, 108 aa, synthetic construct
EIVLTQSPGTLSLSPGERATLSCRASQSVSSSYLAWYQQKPGCAPRLLIYGTSSRATGIPDRFSGSGSGTDFTLTISRLEPEDFAVYYCQAYGSWPITFGQGTRLEIK

SEQ ID NO: 78 - protein, 118 aa, synthetic construct
QVQLQESGPGLVKPSQTLSLTCTVSGGSISSGEYYWNWIRQHPGKGLEWIGYIYYSGSTYYNPSLKSRVTISVDTSKNQFSLKLSSVTAADTAVYYCARESVAGFCYWGQGTLVTVSS

SEQ ID NO: 79 - protein, 108 aa, synthetic construct
EIVLTQSPGTLSLSPGERATLSCRASQSVSSSYLAWYQQKPGQAPRCLIYGTSSRATGIPDRFSGSGSGTDFTLTISRLEPEDFAVYYCQAYGSWPITFGQGTRLEIK

SEQ ID NO: 80 - protein, 118 aa, synthetic construct
QVQLQESGPGLVKPSQTLSLTCTVSGGSISSGEYYWNWIRQHPGKGLEWIGYIYYSGSTYYNPSLKSRVTISVDTSKNQFSLKLSSVTAADTAVYYCARESVAGCDYWGQGTLVTVSS

SEQ ID NO: 81 - protein, 118 aa, synthetic construct
QVQLQESGPGLVKPSQTLSLTCTVSGGSISSGEYYWNWIRQHPGKGLEWIGYIYYSGSTYYNPSLKSRVTISVDTSKNQFSLKLSSVTAADTAVYYCARESVAGFDYCGQGTLVTVSS

SEQ ID NO: 82 - protein, 718 aa, synthetic construct
EVQLVESGGGLVQPGGSLRLSCAASGYTFTNYGMNWVRQAPGKGLEWVGWINTYTGEPTYAADFKRRFTFSLDTSKSTAYLQMNSLRAEDTAVYYCAKYPHYYGSSHWYFDVWGQGTLVTVSSASTKGPSVFPLAPSSKSTSGGTAALGCLVKDYFPEPVTVSWNSGALTSGVHTFPAVLQSSGLYSLSSVVTVPSSSLGTQTYICNVNHKPSNTKVDKKVEPKSCDKTHTCPPCPAPEAAGGPSVFLFPPKPKDTLMISRTPEVTCVVVDVSHEDPEVKFNWYVDGVEVHNAKTKPREEQYNSTYRVVSVLTVLHQDWLNGKEYKCKVSNKALPAPIEKTISKAKGQPREPQVYTLPPSREEMTKNQVSLTCLVKGFYPSDIAVEWESNGQPENNYKTTPPVLDSDGSFFLYSKLTVDKSRWQQGNVFSCSVMHEALHNHYTQKSLSLSPGGGGGSGGGGSGGGGSGGGGSQVQLQESGPGLVKPSQTLSLTCTVSGGSISSGEYYWNWIRQHPGKGLEWIGYIYYSGSTYYNPSLKSRVTISVDTSKNQFSLKLSSVTAADTAVYYCARESVAGFDYCGQGTLVTVSSGGGGSGGGGSGGGGSGGGGSEIVLTQSPGTLSLSPGERATLSCRASQSVSSSYLAWYQQKPGQCPRLLIYGTSSRATGIPDRFSGSGSGTDFTLTISRLEPEDFAVYYCQAYGSWPITFGQGTRLEIK

SEQ ID NO: 83 - protein, 113 aa, synthetic construct [sequence omitted]

SEQ ID NO: 84 - protein, 8 aa, synthetic construct
GITFSNSG

SEQ ID NO: 85 - protein, 8 aa, synthetic construct
IWYDGSKR

SEQ ID NO: 86 - protein, 6 aa, synthetic construct
ATNDDY

SEQ ID NO: 87 - protein, 107 aa, synthetic construct [sequence omitted]

SEQ ID NO: 88 - protein, 6 aa, synthetic construct
QSVSSY

SEQ ID NO: 89 - skipped

SEQ ID NO: 90 - protein, 9 aa, synthetic construct
QQSSNWPRT

SEQ ID NO: 91 - protein, 327 aa, synthetic construct
ASTKGPSVFPLAPCSRSTSESTAALGCLVKDYFPEPVTVSWNSGALTSGVHTFPAVLQSSGLYSLSSVVTVPSSSLGTKTYTCNVDHKPSNTKVDKRVESKYGPPCPPCPAPEFLGGPSVFLFPPKPKDTLMISRTPEVTCVVVDVSQEDPEVQFNWYVDGVEVHNAKTKPREEQFNSTYRVVSVLTVLHQDWLNGKEYKCKVSNKGLPSSIEKTISKAKGQPREPQVYTLPPSQEEMTKNQVSLTCLVKGFYPSDIAVEWESNGQPENNYKTTPPVLDSDGSFFLYSRLTVDKSRWQEGNVFSCSVMHEALHNHYTQKSLSLSLGK

SEQ ID NO: 92 - protein, 107 aa, synthetic construct [sequence omitted]

SEQ ID NO: 93 - protein, 706 aa, synthetic construct
QVQLVESGGGVVQPGRSLRLDCKASGITFSNSGMHWVRQAPGKGLEWVAVIWYDGSKRYYADSVKGRFTISRDNSKNTLFLQMNSLRAEDTAVYYCATNDDYWGQGTLVTVSSASTKGPSVFPLAPCSRSTSESTAALGCLVKDYFPEPVTVSWNSGALTSGVHTFPAVLQSSGLYSLSSVVTVPSSSLGTKTYTCNVDHKPSNTKVDKRVESKYGPPCPPCPAPEFLGGPSVFLFPPKPKDTLMISRTPEVTCVVVDVSQEDPEVQFNWYVDGVEVHNAKTKPREEQFNSTYRVVSVLTVLHQDWLNGKEYKCKVSNKGLPSSIEKTISKAKGQPREPQVYTLPPSQEEMTKNQVSLTCLVKGFYPSDIAVEWESNGQPENNYKTTPPVLDSDGSFFLYSRLTVDKSRWQEGNVFSCSVMHEALHNHYTQKSLSLSLGKGGGGSGGGGSGGGGSGGGGSQVQLQESGPGLVKPSQTLSLTCTVSGGSISSGEYYWNWIRQHPGKCLEWIGYIYYSGSTYYNPSLKSRVTISVDTSKNQFSLKLSSVTAADTAVYYCARESVAGFDYWGQGTLVTVSSGGGGSGGGGSGGGGSGGGGSEIVLTQSPGTLSLSPGERATLSCRASQSVSSSYLAWYQQKPGQAPRLLIYGTSSRATGIPDRFSGSGSGTDFTLTISRLEPEDFAVYYCQAYGSWPITFGCGTRLEIK

SEQ ID NO: 94 - protein, 214 aa, synthetic construct
EIVLTQSPATLSLSPGERATLSCRASQSVSSYLAWYQQKPGQAPRLLIYDASNRATGIPARFSGSGSGTDFTLTISSLEPEDFAVYYCQQSSNWPRTFGQGTKVEIKRTVAAPSVFIFPPSDEQLKSGTASVVCLLNNFYPREAKVQWKVDNALQSGNSQESVTEQDSKDSTYSLSSTLTLSKADYEKHKVYACEVTHQGLSSPVTKSFNRGEC